European Patent Application EP 4 310 101 A1, published January 24, 2024. Title: Novel Anti-nectin-4-Antibodies and Antibody-Drug conjugates. Applicant: Emergence Therapeutics AG. The sequence listing filed with the application follows.

SEQUENCE LISTING (104 sequences)

SEQ ID NO: 1 - protein, 8 aa, synthetic construct
  REGION 1..8: note = CDR1 VH_15A7.5 IMGT
GFTFSNYG

SEQ ID NO: 2 - protein, 8 aa, synthetic construct
  REGION 1..8: note = CDR2 VH_15A7.5 IMGT
ISNLAYGI

SEQ ID NO: 3 - protein, 12 aa, synthetic construct
  REGION 1..12: note = CDR3 VH_15A7.5 IMGT
ARGARATGWFAY

SEQ ID NO: 4 - protein, 6 aa, synthetic construct
  REGION 1..6: note = CDR1 VK_15A7.5 IMGT
QNVDTH

SEQ ID NO: 5 - skipped

SEQ ID NO: 6 - protein, 9 aa, synthetic construct
  REGION 1..9: note = CDR3 VK_15A7.5 IMGT
QQYNSYPLT

SEQ ID NO: 7 - protein, 5 aa, synthetic construct
  REGION 1..5: note = CDR1 VH_15A7.5 Kabat
NYGMA

SEQ ID NO: 8 - protein, 17 aa, synthetic construct
  REGION 1..17: note = CDR2 VH_15A7.5 Kabat
FISNLAYGINYADTVTG

SEQ ID NO: 9 - protein, 10 aa, synthetic construct
  REGION 1..10: note = CDR3 VH_15A7.5 Kabat
GARATGWFAY

SEQ ID NO: 10 - protein, 11 aa, synthetic construct
  REGION 1..11: note = CDR1 VK_15A7.5 Kabat
KASQNVDTHVA

SEQ ID NO: 11 - protein, 7 aa, synthetic construct
  REGION 1..7: note = CDR2 VK_15A7.5 Kabat
SASYRYS

SEQ ID NO: 12 - protein, 9 aa, synthetic construct
  REGION 1..9: note = CDR3 VK_15A7.5 Kabat
QQYNSYPLT

SEQ ID NO: 13 - protein, 119 aa, synthetic construct
  REGION 1..119: note = VH_15A7.5
EVKLVESGGGLVQPGGSRKLSCAASGFTFSNYGMAWVRQAPGKGPEWVAFISNLAYGINYADTVTGRFTISRENAKNTLYLEMRSLRSEDTAMYYCARGARATGWFAYWGQGTLVTVSA

SEQ ID NO: 14 - protein, 107 aa, synthetic construct
  REGION 1..107: note = VK_15A7.5
DIVMTQSQKFMSTSIGDRVSVTCKASQNVDTHVAWYQEKPGQSPKALIYSASYRYSGVPDRFTGSGSGTDFTLTISNVQSEDLADYFCQQYNSYPLTFGGGTKLEIK

SEQ ID NO: 15 - protein, 9 aa, synthetic construct
  REGION 1..9: note = CDR1 H0_15A7.5IMGT
GFTFSNYGM

SEQ ID NO: 16 - protein, 8 aa, synthetic construct
  REGION 1..8: note = CDR2 H0_15A7.5IMGT
ISNLAYGI

SEQ ID NO: 17 - protein, 12 aa, synthetic construct
  REGION 1..12: note = CDR3 H0_15A7.5IMGT
ARGARATGWFAY

SEQ ID NO: 18 - protein, 6 aa, synthetic construct
  REGION 1..6: note = CDR1 L0_15A7.5 IMGT
QNVDTH

SEQ ID NO: 19 - skipped

SEQ ID NO: 20 - protein, 9 aa, synthetic construct
  REGION 1..9: note = CDR3 L0_15A7.5 IMGT
QQYNSYPLT

SEQ ID NO: 21 - protein, 5 aa, synthetic construct
  REGION 1..5: note = CDR1 H0_15A7.5Kabat
NYGMN

SEQ ID NO: 22 - protein, 17 aa, synthetic construct
  REGION 1..17: note = CDR2 H0_15A7.5Kabat
FISNLAYGINYADSVKG

SEQ ID NO: 23 - protein, 10 aa, synthetic construct
  REGION 1..10: note = CDR3 H0_15A7.5Kabat
GARATGWFAY

SEQ ID NO: 24 - protein, 11 aa, synthetic construct
  REGION 1..11: note = CDR1 L0_15A7.5 Kabat
RASQNVDTHVA

SEQ ID NO: 25 - protein, 7 aa, synthetic construct
  REGION 1..7: note = CDR2 L0_15A7.5 Kabat
SASYLQS

SEQ ID NO: 26 - protein, 9 aa, synthetic construct
  REGION 1..9: note = CDR3 L0_15A7.5 Kabat
QQYNSYPLT

SEQ ID NO: 27 - protein, 119 aa, synthetic construct
  REGION 1..119: note = H0_15A7.5
EVQLVESGGGLVQPGGSLRLSCAASGFTFSNYGMNWVRQAPGKGLEWVSFISNLAYGINYADSVKGRFTISRDNAKNSLYLQMNSLRAEDTAVYYCARGARATGWFAYWGQGTLVTVSS

SEQ ID NO: 28 - protein, 107 aa, synthetic construct
  REGION 1..107: note = L0_15A7.5
DIQMTQSPSSLSASVGDRVTITCRASQNVDTHVAWFQQKPGKAPKSLIYSASYLQSGVPSRFSGSGSGTDFTLTISSLQPEDFATYYCQQYNSYPLTFGGGTKVEIK

SEQ ID NO: 29 - protein, 8 aa, synthetic construct
  REGION 1..8: note = CDR1 H1_15A7.5 IMGT
GFTFSNYG

SEQ ID NO: 30 - protein, 8 aa, synthetic construct
  REGION 1..8: note = CDR2 H1_15A7.5 IMGT
ISNLAYGI

SEQ ID NO: 31 - protein, 12 aa, synthetic construct
  REGION 1..12: note = CDR3 H1_15A7.5 IMGT
ARGARATGWFAY

SEQ ID NO: 32 - protein, 6 aa, synthetic construct
  REGION 1..6: note = CDR1 L1_15A7.5 IMGT
QNVDTH

SEQ ID NO: 33 - skipped

SEQ ID NO: 34 - protein, 9 aa, synthetic construct
  REGION 1..9: note = CDR3 L1_15A7.5 IMGT
QQYNSYPLT

SEQ ID NO: 35 - protein, 5 aa, synthetic construct
  REGION 1..5: note = CDR1 H1_15A7.5 Kabat
NYGMA

SEQ ID NO: 36 - protein, 17 aa, synthetic construct
  REGION 1..17: note = CDR2 H1_15A7.5 Kabat
FISNLAYGINYADTVTG

SEQ ID NO: 37 - protein, 10 aa, synthetic construct
  REGION 1..10: note = CDR3 H1_15A7.5 Kabat
GARATGWFAY

SEQ ID NO: 38 - protein, 11 aa, synthetic construct
  REGION 1..11: note = CDR1 L1_15A7.5 Kabat
KASQNVDTHVA

SEQ ID NO: 39 - protein, 7 aa, synthetic construct
  REGION 1..7: note = CDR2 L1_15A7.5 Kabat
SASYRYS

SEQ ID NO: 40 - protein, 9 aa, synthetic construct
  REGION 1..9: note = CDR3 L1_15A7.5 Kabat
QQYNSYPLT

SEQ ID NO: 41 - protein, 119 aa, synthetic construct
  REGION 1..119: note = H1_15A7.5
EVQLVESGGGLVQPGGSLRLSCAASGFTFSNYGMAWVRQAPGKGLEWVSFISNLAYGINYADTVTGRFTISRDNAKNSLYLQMNSLRAEDTAVYYCARGARATGWFAYWGQGTLVTVSS

SEQ ID NO: 42 - protein, 108 aa, synthetic construct
  REGION 1..108: note = L1_15A7.5
DIQMTQSPSSLSASVGDRVTITCCKASQNVDTHVAWFQQKPGKAPKSLIYSASYRYSGVPSRFSGSGSGTDFTLTISSLQPEDFATYYCQQYNSYPLTFGGGTKVEIK

SEQ ID NO: 43 - protein, 8 aa, synthetic construct
  REGION 1..8: note = CDR1 H2_15A7.5 IMGT
GFTFSNYG

SEQ ID NO: 44 - protein, 8 aa, synthetic construct
  REGION 1..8: note = CDR2 H2_15A7.5 IMGT
ISNLAYGI

SEQ ID NO: 45 - protein, 12 aa, synthetic construct
  REGION 1..12: note = CDR3 H2_15A7.5 IMGT
ARGARATGWFAY

SEQ ID NO: 46 - protein, 6 aa, synthetic construct
  REGION 1..6: note = CDR1 L2_15A7.5 IMGT
QNVDTH

SEQ ID NO: 47 - skipped

SEQ ID NO: 48 - protein, 9 aa, synthetic construct
  REGION 1..9: note = CDR3 L2_15A7.5 IMGT
QQYNSYPLT

SEQ ID NO: 49 - protein, 5 aa, synthetic construct
  REGION 1..5: note = CDR1 H2_15A7.5 Kabat
NYGMA

SEQ ID NO: 50 - protein, 17 aa, synthetic construct
  REGION 1..17: note = CDR2 H2_15A7.5 Kabat
FISNLAYGINYADTVTG

SEQ ID NO: 51 - protein, 10 aa, synthetic construct
  REGION 1..10: note = CDR3 H2_15A7.5 Kabat
GARATGWFAY

SEQ ID NO: 52 - protein, 11 aa, synthetic construct
  REGION 1..11: note = CDR1 L2_15A7.5 Kabat
KASQNVDTHVA

SEQ ID NO: 53 - protein, 7 aa, synthetic construct
  REGION 1..7: note = CDR2 L2_15A7.5 Kabat
SASYRYS

SEQ ID NO: 54 - protein, 9 aa, synthetic construct
  REGION 1..9: note = CDR3 L2_15A7.5 Kabat
QQYNSYPLT

SEQ ID NO: 55 - protein, 119 aa, synthetic construct
  REGION 1..119: note = H2_15A7.5
EVQLVESGGGLVQPGGSLRLSCAASGFTFSNYGMAWVRQAPGKGLEWVAFISNLAYGINYADTVTGRFTISRDNAKNSLYLQMNSLRAEDTAVYYCARGARATGWFAYWGQGTLVTVSS

SEQ ID NO: 56 - protein, 107 aa, synthetic construct
  REGION 1..107: note = L2_15A7.5
DIQMTQSPSSLSASVGDRVTITCKASQNVDTHVAWYQQKPGKAPKALIYSASYRYSGVPSRFSGSGSGTDFTLTISSLQPEDFATYYCQQYNSYPLTFGGGTKVEIK

SEQ ID NO: 57 - protein, 8 aa, synthetic construct
  REGION 1..8: note = CDR1 H3_15A7.5 IMGT
GFTFSNYG

SEQ ID NO: 58 - protein, 8 aa, synthetic construct
  REGION 1..8: note = CDR2 H3_15A7.5 IMGT
ISNLAYGI

SEQ ID NO: 59 - protein, 12 aa, synthetic construct
  REGION 1..12: note = CDR3 H3_15A7.5 IMGT
ARGARATGWFAY

SEQ ID NO: 60 - protein, 6 aa, synthetic construct
  REGION 1..6: note = CDR1 L3_15A7.5 IMGT
QNVDTH

SEQ ID NO: 61 - skipped

SEQ ID NO: 62 - protein, 9 aa, synthetic construct
  REGION 1..9: note = CDR3 L3_15A7.5 IMGT
QQYNSYPLT

SEQ ID NO: 63 - protein, 5 aa, synthetic construct
  REGION 1..5: note = CDR1 H3_15A7.5 Kabat
NYGMA

SEQ ID NO: 64 - protein, 17 aa, synthetic construct
  REGION 1..17: note = CDR2 H3_15A7.5 Kabat
FISNLAYGINYADTVTG

SEQ ID NO: 65 - protein, 10 aa, synthetic construct
  REGION 1..10: note = CDR3 H3_15A7.5 Kabat
GARATGWFAY

SEQ ID NO: 66 - protein, 11 aa, synthetic construct
  REGION 1..11: note = CDR1 L3_15A7.5 Kabat
KASQNVDTHVA

SEQ ID NO: 67 - protein, 7 aa, synthetic construct
  REGION 1..7: note = CDR2 L3_15A7.5 Kabat
SASYRYS

SEQ ID NO: 68 - protein, 9 aa, synthetic construct
  REGION 1..9: note = CDR3 L3_15A7.5 Kabat
QQYNSYPLT

SEQ ID NO: 69 - protein, 119 aa, synthetic construct
  REGION 1..119: note = H3_15A7.5
EVQLVESGGGLVQPGGSLRLSCAASGFTFSNYGMAWVRQAPGKGPEWVAFISNLAYGINYADTVTGRFTISRDNAKNSLYLQMNSLRAEDTAVYYCARGARATGWFAYWGQGTLVTVSS

SEQ ID NO: 70 - protein, 108 aa, synthetic construct
  REGION 1..108: note = L3_15A7.5
DIQMTQSPSSLSASVGDRVTITCKASQNVDTHVAWYYQQKPGKSPKALIYSASYRYSGVPSRFSGSGSGTDFTLTISSLQPEDFATYYCQQYNSYPLTFGGGTKVEIK

SEQ ID NO: 71 - protein, 8 aa, synthetic construct
  REGION 1..8: note = CDR1 VH_5A12.2
GFTFNSMY

SEQ ID NO: 72 - protein, 8 aa, synthetic construct
  REGION 1..8: note = CDR2 VH_5A12.2
IYAGTGGT

SEQ ID NO: 73 - protein, 13 aa, synthetic construct
  REGION 1..13: note = CDR3 VH_5A12.2
AIRSGFVPMDYWG

SEQ ID NO: 74 - protein, 118 aa, synthetic construct
  REGION 1..118: note = VH_5A12.2
QIQLQQSGAELVKPGASVTLSCKTSGFTFNSMYISWLKQKPGQSLEWIAWIYAGTGGTRFNQKFTGKVQLTVDTSSSTAYMQFSSLTTDDSAIYYCAIRSGFVPMDYWGQGTSVTVSS

SEQ ID NO: 75 - protein, 6 aa, synthetic construct
  REGION 1..6: note = CDR1 VK_5A12.2
QSVSND

SEQ ID NO: 76 - skipped

SEQ ID NO: 77 - protein, 6 aa, synthetic construct
  REGION 1..6: note = CDR3 VK_5A12.2
QQDYSS

SEQ ID NO: 78 - protein, 107 aa, synthetic construct
  REGION 1..107: note = VK_5A12.2
SIVMTQTPKFLLVSAGDRVTITCKASQSVSNDVAWYQQKPGQSPKLLIYYASNRYTGVPDRFTGSGYGTDFTFTISTVQAEDLAVYFCQQDYSSPWTFGGGTKLEIK

SEQ ID NO: 79 - protein, 8 aa, synthetic construct
  REGION 1..8: note = CDR1 VH_9A2.7
GYNFTTFW

SEQ ID NO: 80 - protein, 8 aa, synthetic construct
  REGION 1..8: note = CDR2 VH_9A2.7
IYPSDSYA

SEQ ID NO: 81 - protein, 13 aa, synthetic construct
  REGION 1..13: note = CDR3 VH_9A2.7
TRPSYFGRNSFAY

SEQ ID NO: 82 - protein, 120 aa, synthetic construct
  REGION 1..120: note = VH_9A2.7
QVQLQQPGAELVRPGASVKLSCKASGYNFTTFWINWVKQRPGQGLEWIGNIYPSDSYANYNQKFKDKATLTVDKSSTTAYMQLSSPTSEDSAVYYCTRPSYFGRNSFAYWGQGTLVTVSA

SEQ ID NO: 83 - protein, 12 aa, synthetic construct
  REGION 1..12: note = CDR1 VK_9A2.7
QSLLYSVNHKNY

SEQ ID NO: 84 - skipped

SEQ ID NO: 85 - protein, 9 aa, synthetic construct
  REGION 1..9: note = CDR3 VK_9A2.7
HQYYTYPLT

SEQ ID NO: 86 - protein, 113 aa, synthetic construct
  REGION 1..113: note = VK_9A2.7
DIVMTQSPSSLVVSVGEKVTMSCKSSQSLLYSVNHKNYLAWYQQKPGQSPKLLIYWASTRESGVPDRFTGSGSGTDFSLTISSVKAEDLAVYYCHQYYTYPLTFGAGTKLELK

SEQ ID NO: 87 - protein, 8 aa, synthetic construct
  REGION 1..8: note = CDR1 VH_3A1.4
GDSITSGY

SEQ ID NO: 88 - protein, 7 aa, synthetic construct
  REGION 1..7: note = CDR2 VH_3A1.4
ISNSGIT

SEQ ID NO: 89 - protein, 15 aa, synthetic construct
  REGION 1..15: note = CDR3 VH_3A1.4
TRFGSTMILYYTMDY

SEQ ID NO: 90 - protein, 121 aa, synthetic construct
  REGION 1..121: note = VH_3A1.4
DVQLQESGPSLVKPSQTLSLTCSVTGDSITSGYWNWIRKFPGNKLEYMGYISNSGITYYNPSLKSRISITRDTSKNQYFLQLNSVTAEDTATYYCTRFGSTMILYYTMDYWGQGTSVTVSS

SEQ ID NO: 91 - protein, 6 aa, synthetic construct
  REGION 1..6: note = CDR1 VK_3A1.4
QSISDY

SEQ ID NO: 92 - skipped

SEQ ID NO: 93 - protein, 9 aa, synthetic construct
  REGION 1..9: note = CDR3 VK_3A1.4
QNGHSFPLT

SEQ ID NO: 94 - protein, 107 aa, synthetic construct
  REGION 1..107: note = VK_3A1.4
DIVMTQSPVTLSVTPGDRVSLSCRASQSISDYLHWYQQKSQESPRLLIKYASKSISGIPSRFSGSGSGSNFTLSINSVEPEDVGVYYCQNGHSFPLTFGAGTKLELK

SEQ ID NO: 95 - protein, 8 aa, synthetic construct
  REGION 1..8: note = CDR1 VH_8F06
GYTFTSYV

SEQ ID NO: 96 - protein, 8 aa, synthetic construct
  REGION 1..8: note = CDR2 VH_8F06
INPYNDGT

SEQ ID NO: 97 - protein, 6 aa, synthetic construct
  REGION 1..6: note = CDR3 VH_8F06
VTLFAY

SEQ ID NO: 98 - protein, 113 aa, synthetic construct
  REGION 1..113: note = VH_8F06
EVQLQQSGPELVKPGASVKMSCKASGYTFTSYVMHWVKQKPGQGLEWIGYINPYNDGTKYNEKFKGKATLTSDKSSSTAYMELSSLTSEDSAVYYCVTLFAYWGQGTLVTVSA

SEQ ID NO: 99 - protein, 5 aa, synthetic construct
  REGION 1..5: note = CDR1 VK_8F06
SSISY

SEQ ID NO: 100 - skipped

SEQ ID NO: 101 - protein, 9 aa, synthetic construct
  REGION 1..9: note = CDR3 VK_8F06
HQRSSYPFT

SEQ ID NO: 102 - protein, 106 aa, synthetic construct
  REGION 1..106: note = VK_8F06
QIVLTQSPAIMSASPGEKVTMTCSASSSISYMHWYQQKPGTSPKRWIYDTSKLASGVPARFSGSGSGTSYSLTISSMEAEDAATYYCHQRSSYPFTFGSGTKLEIK

SEQ ID NO: 103 - protein, 107 aa, synthetic construct
  REGION 1..107: note = L3_15A7.5_mod
DIQMTQSPSSLSASVGDRVTITCKASQNVDTHVAWYYQQKPGKSPKALIYSASYRYSGVPSRFSGSGSGTDFTLTISSLQPEDFATYCQQYNSYPLTFGGGTKVEIK

SEQ ID NO: 104 - protein, 510 aa, unidentified
MPLSLGAEMWGPEAWLLLLLLLASFTGRCPAGELETSDVVTVVLGQDAKLPCFYRGDSGEQVGQVAWARVDAGEGAQELALLHSKYGLHVSPAYEGRVEQPPPPRNPLDGSVLLRNAVQADEGEYECRVSTFPAGSFQARLRLRVLVPPLPSLNPGPALEEGQGLTLAASCTAEGSPAPSVTWDTEVKGTTSSRSFKHSRSAAVTSEFHLVPSRSMNGQPLTCVVSHPGLLQDQRITHILHVSFLAEASVRGLEDQNLWHIGREGAMLKCLSEGQPPPSYNWTRLDGPLPSGVRVDGDTLGFPPLTTEHSGIYVCHVSNEFSSRDSQVTVDVLDPQEDSGKQVDLVSASVVVVGVIAALLFCLLVVVVVLMSRYHRRKAQQMTQKYEEELTLTRENSIRRLHSHHTDPRSQPEESVGLRAEGHPDSLKDNSSCSVMSEEPEGRSYSTLTTVREIETQTELLSPGSGRAEEEEDQDEGIKQAMNHFVQENGTLRAKPTGNGIYINGRGHLV